European Patent Specification EP 3 299 382 B1, published April 26, 2023. Title: Drug for preventing or treating infarction. Applicant: OSAKA UNIVERSITY. The sequence listing filed with the application follows.

SEQUENCE LISTING (24 sequences)

SEQ ID NO: 1 - protein, 7 aa, Homo sapiens
SIKIPSS

SEQ ID NO: 2 - protein, 8 aa, Mus musculus
LMVYVVKT

SEQ ID NO: 3 - protein, 11 aa, Mus musculus
YLQLMVYVVKT

SEQ ID NO: 4 - protein, 8 aa, Homo sapiens
LMVYVTKT

SEQ ID NO: 5 - protein, 11 aa, Homo sapiens
YLQLMVYVTKT

SEQ ID NO: 6 - protein, 9 aa, Mus musculus
HNLMKGGST

SEQ ID NO: 7 - protein, 7 aa, Mus musculus
HNLMKGG

SEQ ID NO: 8 - protein, 9 aa, Homo sapiens
HTLMKGGST

SEQ ID NO: 9 - protein, 7 aa, Homo sapiens
HTLMKGG

SEQ ID NO: 10 - protein, 30 aa, Mus musculus
LMVYVVKTSIKIPSSHNLMKGGSTKNWSGN

SEQ ID NO: 11 - protein, 30 aa, Mus musculus
DYLQLMVYVVKTSIKIPSSHNLMKGGSTKN

SEQ ID NO: 12 - protein, 15 aa, Mus musculus
LMVYVVKTSIKIPSS

SEQ ID NO: 13 - protein, 22 aa, Mus musculus
LMVYVVKTSIKIPSSHNLMKGG

SEQ ID NO: 14 - protein, 30 aa, Homo sapiens
LMVYVTKTSIKIPSSHTLMKGGSTKYWSGN

SEQ ID NO: 15 - protein, 10 aa, Mus musculus
HETSGSVPAD

SEQ ID NO: 16 - protein, 10 aa, Homo sapiens
HETSGDLATE

SEQ ID NO: 17 - DNA, 23 bp, Artificial Sequence
  RANK siRNA sequence
gcgcagacuucacuccauauutt

SEQ ID NO: 18 - DNA, 23 bp, Artificial Sequence
  RANK siRNA sequence
uauggagugaagucugcgcuutt

SEQ ID NO: 19 - DNA, 23 bp, Artificial Sequence
  control siRNA sequence
uagcgacuaaacacaucaauutt

SEQ ID NO: 20 - DNA, 23 bp, Artificial Sequence
  control siRNA sequence
uuaucgcugauuuguguaguutt

SEQ ID NO: 21 - protein, 28 aa, Mus musculus
HETSGSVPADYLQLMVYVVKTSIKIPSS

SEQ ID NO: 22 - protein, 23 aa, Mus musculus
LMVYVVKTSIKIPSSHNLMKGGS

SEQ ID NO: 23 - protein, 26 aa, Mus musculus
LMVYVVKTSIKIPSSHNLMKGGSTKN

SEQ ID NO: 24 - protein, 11 aa, Mus musculus
LMVYVVKTSIK